European Patent Application EP 4 803 628 A1, published September 9, 2026. Title: Aptamers for nuclear translocation. Applicant: TYRIS THERAPEUTICS, S.L. Application EP. The sequence listing filed with the application follows.

SEQUENCE LISTING (176 sequences)

SEQ ID NO: 1 - DNA, 45 bp, Synthetic construct
  source 1..45: mol_type = other DNA
ccgcctgtgtcttacctaatgttgcgtcatctctgtgcgtcacga

SEQ ID NO: 2 - DNA, 45 bp, Synthetic construct
  source 1..45: mol_type = other DNA
gcacaccacatcatactgtgtccaaccgttttgcgagtcctcccg

SEQ ID NO: 3 - DNA, 45 bp, Synthetic construct
  source 1..45: mol_type = other DNA
tggtgtgtgtgcttatccctttctttggtcggttgctgcgttttg

SEQ ID NO: 4 - DNA, 45 bp, Synthetic construct
  source 1..45: mol_type = other DNA
caaaccacgacataccttttccgttccaggcaggtctttattccg

SEQ ID NO: 5 - DNA, 45 bp, Synthetic construct
  source 1..45: mol_type = other DNA
ccccaccgctcaccatagtcactctcattgtccaacctctcactc

SEQ ID NO: 6 - DNA, 45 bp, Synthetic construct
  source 1..45: mol_type = other DNA
ccacacatccaaccgtaaatgctccttgtccagcaacccttaccg

SEQ ID NO: 7 - DNA, 45 bp, Synthetic construct
  source 1..45: mol_type = other DNA
caacacacatttcctcccccggcactgctggtcgattcgcgcggt

SEQ ID NO: 8 - DNA, 45 bp, Synthetic construct
  source 1..45: mol_type = other DNA
ggttatgtgggtggtgctgctgtgatggtgatgcgtccgatgggg

SEQ ID NO: 9 - DNA, 45 bp, Synthetic construct
  source 1..45: mol_type = other DNA
cacaactgaacacattgctgcacgtcttgatccctagctggttgc

SEQ ID NO: 10 - DNA, 45 bp, Synthetic construct
  source 1..45: mol_type = other DNA
acaacgcctctcttcttcttgccctgagaacacacacactacccg

SEQ ID NO: 11 - DNA, 45 bp, Synthetic construct
  source 1..45: mol_type = other DNA
acacacaccatgcttctttgccctttctctcttttgcttcccctg

SEQ ID NO: 12 - DNA, 45 bp, Synthetic construct
  source 1..45: mol_type = other DNA
acaacaattacccgtagtccagcatccgacgttctcctgccctcg

SEQ ID NO: 13 - DNA, 45 bp, Synthetic construct
  source 1..45: mol_type = other DNA
ccaccaacactcgtcatgctttggtcatctctgccccatgctgcg

SEQ ID NO: 14 - DNA, 45 bp, Synthetic construct
  source 1..45: mol_type = other DNA
aacccaccactcactctgcttgtttgcccgatgctgccctacctg

SEQ ID NO: 15 - DNA, 45 bp, Synthetic construct
  source 1..45: mol_type = other DNA
accaactcgcgtcctcacaacctgtctgcgtcctttcccatgctg

SEQ ID NO: 16 - DNA, 45 bp, Synthetic construct
  source 1..45: mol_type = other DNA
cagtgcgttatcccatgctgcgtttcaacatgatgcgtcttcgtg

SEQ ID NO: 17 - DNA, 45 bp, Synthetic construct
  source 1..45: mol_type = other DNA
acaccacacaccacacaccactcctgatctttgggactcgcctgt

SEQ ID NO: 18 - DNA, 45 bp, Synthetic construct
  source 1..45: mol_type = other DNA
cacaggcgatcatcactgctgctgtctatcattatgctgcgttcg

SEQ ID NO: 19 - DNA, 45 bp, Synthetic construct
  source 1..45: mol_type = other DNA
caacatcatcacgtgtccagtctatgctgctgcttcccccttccg

SEQ ID NO: 20 - DNA, 45 bp, Synthetic construct
  source 1..45: mol_type = other DNA
accccctgctgtcatttgtgcaagtcacttattcgctgcgcacga

SEQ ID NO: 21 - DNA, 45 bp, Synthetic construct
  source 1..45: mol_type = other DNA
ccggtccaaatccccaacgtgttttgttgctgccttttgtccccg

SEQ ID NO: 22 - DNA, 45 bp, Synthetic construct
  source 1..45: mol_type = other DNA
acaccaaactgcacatcttgcttgtgtccagcccctatgtatccg

SEQ ID NO: 23 - DNA, 45 bp, Synthetic construct
  source 1..45: mol_type = other DNA
cccatacgtgtccaacctttcccacaatgtgctgtcgttataccg

SEQ ID NO: 24 - DNA, 45 bp, Synthetic construct
  source 1..45: mol_type = other DNA
ccgtgtctgtctgttatacgtgtccatacaaaacactctggatcg

SEQ ID NO: 25 - DNA, 45 bp, Synthetic construct
  source 1..45: mol_type = other DNA
cacacacaatgagcgtcaatcgtatctttcaaatcttgctgcgtc

SEQ ID NO: 26 - DNA, 45 bp, Synthetic construct
  source 1..45: mol_type = other DNA
cgcacacaatctacctgtccataccgcacaccttctgttactccg

SEQ ID NO: 27 - DNA, 45 bp, Synthetic construct
  source 1..45: mol_type = other DNA
ccacgcattgtccaccgcagcacaattcactatttaccttccccg

SEQ ID NO: 28 - DNA, 45 bp, Synthetic construct
  source 1..45: mol_type = other DNA
tcactaatactgaccgtggacacattacactctggaggatcactc

SEQ ID NO: 29 - DNA, 45 bp, Synthetic construct
  source 1..45: mol_type = other DNA
acacatcatgcttaccctttacctgtccacaacctcccgttactc

SEQ ID NO: 30 - DNA, 45 bp, Synthetic construct
  source 1..45: mol_type = other DNA
ccaccccacatgatcgtccctctgatcgtcactccttactgctgt

SEQ ID NO: 31 - DNA, 45 bp, Synthetic construct
  source 1..45: mol_type = other DNA
gatgtcgacgcaccgttccacaccattcttttcctccatgcactc

SEQ ID NO: 32 - DNA, 45 bp, Synthetic construct
  source 1..45: mol_type = other DNA
tcaacccacattacactgtgtctacccgcccacattccttccctc

SEQ ID NO: 33 - DNA, 45 bp, Synthetic construct
  source 1..45: mol_type = other DNA
ccacacccatatgctgttttgtccaggcgatcaaacgtctcacgg

SEQ ID NO: 34 - DNA, 45 bp, Synthetic construct
  source 1..45: mol_type = other DNA
ggccgtcgcgaaaccatgatgtctgtcactctcatcgcgttactc

SEQ ID NO: 35 - DNA, 45 bp, Synthetic construct
  source 1..45: mol_type = other DNA
acacacactttctcactgcctcttttccctgctctcgcattcggt

SEQ ID NO: 36 - DNA, 45 bp, Synthetic construct
  source 1..45: mol_type = other DNA
gcataatcctcaccgtccacgaacaaattctttcgcactctggta

SEQ ID NO: 37 - DNA, 45 bp, Synthetic construct
  source 1..45: mol_type = other DNA
gccaatccgttcgcactgtgaccagacgccctttactcatatccg

SEQ ID NO: 38 - DNA, 45 bp, Synthetic construct
  source 1..45: mol_type = other DNA
gcagatcgtaccattttcgtccaaccgcgcataacctccttaccg

SEQ ID NO: 39 - DNA, 45 bp, Synthetic construct
  source 1..45: mol_type = other DNA
cccgacaacatgctgcttcttttgtactgtgcgtcactagatggt

SEQ ID NO: 40 - DNA, 45 bp, Synthetic construct
  source 1..45: mol_type = other DNA
acaatggctgtatcccacctgtccacacattcttgtcactctgcc

SEQ ID NO: 41 - DNA, 45 bp, Synthetic construct
  source 1..45: mol_type = other DNA
cgatcccacgcatattacatgtcactctgtttccgtcgctctggt

SEQ ID NO: 42 - DNA, 45 bp, Synthetic construct
  source 1..45: mol_type = other DNA
tggggggttgcttgcgttctggtatgttgttgctgcgttgagtgc

SEQ ID NO: 43 - DNA, 45 bp, Synthetic construct
  source 1..45: mol_type = other DNA
cgatcgtaggtgtggtgatgctgcctttttatgctgcgtccgacg

SEQ ID NO: 44 - DNA, 45 bp, Synthetic construct
  source 1..45: mol_type = other DNA
atacccggtccgatgctgcttacttctttgtcggtgatgcgtcta

SEQ ID NO: 45 - DNA, 45 bp, Synthetic construct
  source 1..45: mol_type = other DNA
tgaccctctctcgtgtccagccttattccttgctgtcgacctccg

SEQ ID NO: 46 - DNA, 45 bp, Synthetic construct
  source 1..45: mol_type = other DNA
cacacacacacgcatctcaacttgctgtcatcttctcccttaccg

SEQ ID NO: 47 - DNA, 45 bp, Synthetic construct
  source 1..45: mol_type = other DNA
gcacatcctcacatacttttgtccagcaaccaacacttcattccg

SEQ ID NO: 48 - DNA, 45 bp, Synthetic construct
  source 1..45: mol_type = other DNA
gggatacgtggttgctgcttatggtgggtgctgcactttaacttg

SEQ ID NO: 49 - DNA, 45 bp, Synthetic construct
  source 1..45: mol_type = other DNA
tgccatcctgtccaccatgtctctgagaaggtgctgcgtattgta

SEQ ID NO: 50 - DNA, 45 bp, Synthetic construct
  source 1..45: mol_type = other DNA
aacaccccactgccacttgtcctttgtcggtgctgcgttttggcg

SEQ ID NO: 51 - DNA, 45 bp, Synthetic construct
  source 1..45: mol_type = other DNA
acatcataacagtgtccaaccccgatattcactcattgttacccg

SEQ ID NO: 52 - DNA, 45 bp, Synthetic construct
  source 1..45: mol_type = other DNA
accaactcgcgtcctcacaacctgtctgcgtcttttcccatgctg

SEQ ID NO: 53 - DNA, 44 bp, Synthetic construct
  source 1..44: mol_type = other DNA
cacgctccatgctcgttcactaccgaaatgcacgttactctgtg

SEQ ID NO: 54 - DNA, 45 bp, Synthetic construct
  source 1..45: mol_type = other DNA
ccaccgtcgacattctgataccgtcactctttcctactgctgcgg

SEQ ID NO: 55 - DNA, 44 bp, Synthetic construct
  source 1..44: mol_type = other DNA
ccccgaacatgctgccaccttattgttgctcccatgctgcacta

SEQ ID NO: 56 - DNA, 45 bp, Synthetic construct
  source 1..45: mol_type = other DNA
caacatcatcacgtgtccagtctatgctgctgctttccccttccg

SEQ ID NO: 57 - DNA, 44 bp, Synthetic construct
  source 1..44: mol_type = other DNA
gggatggtccaccacacacacactctttttgcctccatttgacg

SEQ ID NO: 58 - DNA, 45 bp, Synthetic construct
  source 1..45: mol_type = other DNA
cgtgtccagaccgattttatcccaaactgctgcccctactacgcg

SEQ ID NO: 59 - DNA, 45 bp, Synthetic construct
  source 1..45: mol_type = other DNA
acaaacacatcctcctctttgtccacaaaacactcattctcatcg

SEQ ID NO: 60 - DNA, 45 bp, Synthetic construct
  source 1..45: mol_type = other DNA
ccaaccatgccttgattgtcactctctcttgctgcgtctaccgac

SEQ ID NO: 61 - DNA, 45 bp, Synthetic construct
  source 1..45: mol_type = other DNA
tgaccttaacgtgtccacccacaaaatgtctcgtccttcctactc

SEQ ID NO: 62 - DNA, 45 bp, Synthetic construct
  source 1..45: mol_type = other DNA
cacattgcccttcgttaccgttccacccaacccctttatcacccg

SEQ ID NO: 63 - DNA, 45 bp, Synthetic construct
  source 1..45: mol_type = other DNA
acaccgaacgcttttgatcttgtgtccaagcgcgccttccttccg

SEQ ID NO: 64 - DNA, 45 bp, Synthetic construct
  source 1..45: mol_type = other DNA
ccaccctcactccatgctcgcgtctaaattgcatgttgttgcgcc

SEQ ID NO: 65 - DNA, 45 bp, Synthetic construct
  source 1..45: mol_type = other DNA
cctcgccccatgccttgtcacttcatcatcgtctattgctgcgtt

SEQ ID NO: 66 - DNA, 45 bp, Synthetic construct
  source 1..45: mol_type = other DNA
acaccgttccacaagtcctcctccaccgtttcaacctcttcactc

SEQ ID NO: 67 - DNA, 45 bp, Synthetic construct
  source 1..45: mol_type = other DNA
gccgcatccaccgttccacctcaccccgttttccttgatgccatc

SEQ ID NO: 68 - DNA, 45 bp, Synthetic construct
  source 1..45: mol_type = other DNA
acccaccccgtatcttcgtgtccaccacccttcactctttaccct

SEQ ID NO: 69 - DNA, 45 bp, Synthetic construct
  source 1..45: mol_type = other DNA
cacaggcgatcatcactgctgctgtctatcatcatgctgcgttcg

SEQ ID NO: 70 - DNA, 45 bp, Synthetic construct
  source 1..45: mol_type = other DNA
acacccgatactgtgtccaaccgcaatcctttgttaactcatccg

SEQ ID NO: 71 - DNA, 45 bp, Synthetic construct
  source 1..45: mol_type = other DNA
taggcacctgtccatccaacattcagtcactctatctcatgcacg

SEQ ID NO: 72 - DNA, 45 bp, Synthetic construct
  source 1..45: mol_type = other DNA
aacaccacctcaccactgtagtccatcaccatccgtctatctccg

SEQ ID NO: 73 - DNA, 45 bp, Synthetic construct
  source 1..45: mol_type = other DNA
cacacacacacttcggcatttgtctattctctctttttggtcggg

SEQ ID NO: 74 - DNA, 45 bp, Synthetic construct
  source 1..45: mol_type = other DNA
acccgaactactatcccgttggtccacaaccgcgaatattccccc

SEQ ID NO: 75 - DNA, 45 bp, Synthetic construct
  source 1..45: mol_type = other DNA
ccccgccatgcctttatctgtcatctctgatttctgctgctgcgt

SEQ ID NO: 76 - DNA, 45 bp, Synthetic construct
  source 1..45: mol_type = other DNA
ccacacaccacacatgctctcgtacttgaccttctcgcgaactgg

SEQ ID NO: 77 - DNA, 45 bp, Synthetic construct
  source 1..45: mol_type = other DNA
tggcccacaccttctgtctgtccacacacacattctcctcgtttc

SEQ ID NO: 78 - DNA, 45 bp, Synthetic construct
  source 1..45: mol_type = other DNA
caaccacatgctgttttacacaaacctcgcgccatttctctcacg

SEQ ID NO: 79 - DNA, 45 bp, Synthetic construct
  source 1..45: mol_type = other DNA
acgtggccaccaaagctcattgtgtccaaccctttatcctatccg

SEQ ID NO: 80 - DNA, 45 bp, Synthetic construct
  source 1..45: mol_type = other DNA
ccgtgccaaccctgttatttactcgtgttgttgctcgtcgtcccg

SEQ ID NO: 81 - DNA, 45 bp, Synthetic construct
  source 1..45: mol_type = other DNA
acaaacacaccatgctgcattttcgactgtgcgtctttctgtagt

SEQ ID NO: 82 - DNA, 45 bp, Synthetic construct
  source 1..45: mol_type = other DNA
ccagctgcactcgtcatgctcgtcacgtgtttgctgctcacgttg

SEQ ID NO: 83 - DNA, 45 bp, Synthetic construct
  source 1..45: mol_type = other DNA
cagcccatgcattgattagtgtccagacccagtaccgttccatcg

SEQ ID NO: 84 - DNA, 45 bp, Synthetic construct
  source 1..45: mol_type = other DNA
ccgcccactgctcgtcatagactctttgttgctgcgttgttaatg

SEQ ID NO: 85 - DNA, 45 bp, Synthetic construct
  source 1..45: mol_type = other DNA
gacaacatctcgtgtccaaagcccgattcgaccctttgttttccg

SEQ ID NO: 86 - DNA, 45 bp, Synthetic construct
  source 1..45: mol_type = other DNA
ccgaactccatgctgtcctcgtcattgttgctgctgactcttcgt

SEQ ID NO: 87 - DNA, 45 bp, Synthetic construct
  source 1..45: mol_type = other DNA
acaatggccgtatcccacctgtccacacattcttgtcactctgcc

SEQ ID NO: 88 - DNA, 45 bp, Synthetic construct
  source 1..45: mol_type = other DNA
tcaccacacacacgctttcatggcttctccctatgcatcctcgac

SEQ ID NO: 89 - DNA, 45 bp, Synthetic construct
  source 1..45: mol_type = other DNA
cctcacgcgtacccatgctgctatatccgtcatgctgcttatcgt

SEQ ID NO: 90 - DNA, 45 bp, Synthetic construct
  source 1..45: mol_type = other DNA
accgtgatgtctgttcgtgtccaaaccttttccattctgtctccg

SEQ ID NO: 91 - DNA, 45 bp, Synthetic construct
  source 1..45: mol_type = other DNA
ccgtggacagtcccaccttatcgtctgtctccgtcattctgcccg

SEQ ID NO: 92 - DNA, 45 bp, Synthetic construct
  source 1..45: mol_type = other DNA
tatgttcggggttaacgtgtccaaccaccattgtcatctcctccg

SEQ ID NO: 93 - DNA, 45 bp, Synthetic construct
  source 1..45: mol_type = other DNA
cacacacctgcccctcttgatcacatctcgttgctgcggtttggg

SEQ ID NO: 94 - DNA, 45 bp, Synthetic construct
  source 1..45: mol_type = other DNA
ccacaacccgactgctcgtccaatcttgctgtcactcttggttgg

SEQ ID NO: 95 - DNA, 45 bp, Synthetic construct
  source 1..45: mol_type = other DNA
tggggctgagtgcgtcatcttccatggcttagttgctgcgtttgg

SEQ ID NO: 96 - DNA, 45 bp, Synthetic construct
  source 1..45: mol_type = other DNA
cacaaccaacacaacatcgtcacctcgtattcccactctcgatgc

SEQ ID NO: 97 - DNA, 45 bp, Synthetic construct
  source 1..45: mol_type = other DNA
accgctcaaaacccatgctgctcgtatacaactgcctgctgctcc

SEQ ID NO: 98 - DNA, 45 bp, Synthetic construct
  source 1..45: mol_type = other DNA
tctcccaccccctgctgcttttgacaatgctgctctgatcgttga

SEQ ID NO: 99 - DNA, 45 bp, Synthetic construct
  source 1..45: mol_type = other DNA
tggcgaggattggtgatgcgtcctattatgcgtgctgcttcatcg

SEQ ID NO: 100 - DNA, 45 bp, Synthetic construct
  source 1..45: mol_type = other DNA
ccgccaccaccttactttgtcactcctgatatgtctgctgcggtt

SEQ ID NO: 101 - DNA, 45 bp, Synthetic construct
  source 1..45: mol_type = other DNA
cacaccaaacgcccgccttatactcactctgttgccctgctgctc

SEQ ID NO: 102 - DNA, 45 bp, Synthetic construct
  source 1..45: mol_type = other DNA
caacacaccactcagtgtccaaacgtctcatttatcgtcactccg

SEQ ID NO: 103 - DNA, 45 bp, Synthetic construct
  source 1..45: mol_type = other DNA
ccctctcagaccatttgctgttccctcagtcacgtcatgctgctc

SEQ ID NO: 104 - DNA, 45 bp, Synthetic construct
  source 1..45: mol_type = other DNA
ccacatactcctgtcccgtcaactcgcttctaaccctgctgcgcc

SEQ ID NO: 105 - DNA, 45 bp, Synthetic construct
  source 1..45: mol_type = other DNA
ccacacatgctgatcatcattttcgcgcactcctttcctgctgcc

SEQ ID NO: 106 - DNA, 45 bp, Synthetic construct
  source 1..45: mol_type = other DNA
tcgcccccctaagccacataccctgctcgtcactcactcgtcacg

SEQ ID NO: 107 - DNA, 45 bp, Synthetic construct
  source 1..45: mol_type = other DNA
ccccaacataatgtctctctggcacatgctgcgttagatgttgtg

SEQ ID NO: 108 - DNA, 45 bp, Synthetic construct
  source 1..45: mol_type = other DNA
cagaacaaatgataatcgtgtccagccaatcccacttcctttccg

SEQ ID NO: 109 - DNA, 45 bp, Synthetic construct
  source 1..45: mol_type = other DNA
gcgaaatccccccatgctgtattgcccgaccatctgcgtcttccg

SEQ ID NO: 110 - DNA, 45 bp, Synthetic construct
  source 1..45: mol_type = other DNA
tggggacaggtgctgcttaaattatttgggatgctgcgctgtagt

SEQ ID NO: 111 - DNA, 45 bp, Synthetic construct
  source 1..45: mol_type = other DNA
taatgtacgtgtccaacccaatgctttatggcccacacaaatccg

SEQ ID NO: 112 - DNA, 45 bp, Synthetic construct
  source 1..45: mol_type = other DNA
acccccatgctgttcccttatgtcctgctgtgttttttgtctacg

SEQ ID NO: 113 - DNA, 45 bp, Synthetic construct
  source 1..45: mol_type = other DNA
cgcgccatcacctttgcttcgttactctccgtcaatgctgcggtt

SEQ ID NO: 114 - DNA, 45 bp, Synthetic construct
  source 1..45: mol_type = other DNA
tccccacaccacgatcttcacttttcgctcactctgtcgtacggc

SEQ ID NO: 115 - DNA, 45 bp, Synthetic construct
  source 1..45: mol_type = other DNA
tgaccataaccgcattgtcaattgtccacaccctttcactctgac

SEQ ID NO: 116 - DNA, 45 bp, Synthetic construct
  source 1..45: mol_type = other DNA
caccgattccagcacaacttggcatttgcgtcatctccctcactc

SEQ ID NO: 117 - DNA, 45 bp, Synthetic construct
  source 1..45: mol_type = other DNA
ccccacccacatctgtcgtcgttgttgctgttgttttggtttgtg

SEQ ID NO: 118 - DNA, 45 bp, Synthetic construct
  source 1..45: mol_type = other DNA
taccaacaccctccacctgccaacacaaccctttatgtctcatcg

SEQ ID NO: 119 - DNA, 45 bp, Synthetic construct
  source 1..45: mol_type = other DNA
tgtcccacacatcatcaccttgtccaagcgcgtttgtccttaccg

SEQ ID NO: 120 - DNA, 45 bp, Synthetic construct
  source 1..45: mol_type = other DNA
tcggacccatcccaccgtgccatactacacacattttctcctccg

SEQ ID NO: 121 - DNA, 45 bp, Synthetic construct
  source 1..45: mol_type = other DNA
acacgcaacttctcatagtgtccacccaacttctcgctcactacc

SEQ ID NO: 122 - DNA, 45 bp, Synthetic construct
  source 1..45: mol_type = other DNA
ggaccaccgttgtaccaaacccagctttcatcggcactctgatcg

SEQ ID NO: 123 - DNA, 45 bp, Synthetic construct
  source 1..45: mol_type = other DNA
ccacgctttaccaccaatcacactgctgctcctggttttcgatgc

SEQ ID NO: 124 - DNA, 45 bp, Synthetic construct
  source 1..45: mol_type = other DNA
cgacgccataatgctgctgttcttgatacctgctgcggttgggac

SEQ ID NO: 125 - DNA, 45 bp, Synthetic construct
  source 1..45: mol_type = other DNA
caacatcaagcatctcaccatctgtccagacgttttgccttcccg

SEQ ID NO: 126 - DNA, 45 bp, Synthetic construct
  source 1..45: mol_type = other DNA
acacccacccaatgctttaactttgccttttccacaattcgcggt

SEQ ID NO: 127 - DNA, 45 bp, Synthetic construct
  source 1..45: mol_type = other DNA
gggatcagtccgtgtccaccaattttcctattgtcacttccactc

SEQ ID NO: 128 - DNA, 45 bp, Synthetic construct
  source 1..45: mol_type = other DNA
ggcccagtactttccaccgtccatccgaccctattctatttaccg

SEQ ID NO: 129 - DNA, 45 bp, Synthetic construct
  source 1..45: mol_type = other DNA
cgatgcacaacctgccgatgcgtccttttgttgtttgctgcggtg

SEQ ID NO: 130 - DNA, 45 bp, Synthetic construct
  source 1..45: mol_type = other DNA
cacacatcaccatgctgttttgttaaggttgtcgtacatgcgggt

SEQ ID NO: 131 - DNA, 45 bp, Synthetic construct
  source 1..45: mol_type = other DNA
cacaccacgctatatgcacacacaactcaatcttattatcgcggt

SEQ ID NO: 132 - DNA, 45 bp, Synthetic construct
  source 1..45: mol_type = other DNA
accgaccaacatgctgctcatcaatcctgttctcctcgatcctgc

SEQ ID NO: 133 - DNA, 45 bp, Synthetic construct
  source 1..45: mol_type = other DNA
acaacaattacccgtagtccagcatccgacgttctcttgccctcg

SEQ ID NO: 134 - DNA, 45 bp, Synthetic construct
  source 1..45: mol_type = other DNA
ccaccgccatgctggtttcctcgttcgatgctgatcttgttgggg

SEQ ID NO: 135 - DNA, 45 bp, Synthetic construct
  source 1..45: mol_type = other DNA
gtggtgggtgtgctgtttcactggtttctatggtgtggtgcgtcc

SEQ ID NO: 136 - DNA, 45 bp, Synthetic construct
  source 1..45: mol_type = other DNA
cacacacacacgcccttccatttacgagtttgacttactccctcc

SEQ ID NO: 137 - DNA, 45 bp, Synthetic construct
  source 1..45: mol_type = other DNA
gggtgtgtgctgacttagttttgttgctgctctttttgtgcggtc

SEQ ID NO: 138 - DNA, 45 bp, Synthetic construct
  source 1..45: mol_type = other DNA
cactgccccatgctggtcttgttgaaacatgctgcgttttcatcg

SEQ ID NO: 139 - DNA, 45 bp, Synthetic construct
  source 1..45: mol_type = other DNA
gcacatcctcacatacctttgtccagcaaccaacacttcattccg

SEQ ID NO: 140 - DNA, 45 bp, Synthetic construct
  source 1..45: mol_type = other DNA
cccacattaccgaacccactgtccaaaagcatgtttcgttctccg

SEQ ID NO: 141 - DNA, 45 bp, Synthetic construct
  source 1..45: mol_type = other DNA
cacaccaccattgctgtttttgacctggaacgacttgcatgcggc

SEQ ID NO: 142 - DNA, 45 bp, Synthetic construct
  source 1..45: mol_type = other DNA
taccatacttcacctgtccaccaacccacaccctatacgccctcg

SEQ ID NO: 143 - DNA, 45 bp, Synthetic construct
  source 1..45: mol_type = other DNA
gccaaccacgccatacatgctgtcttttgatttgtgatgcgtccg

SEQ ID NO: 144 - DNA, 45 bp, Synthetic construct
  source 1..45: mol_type = other DNA
ttaccacccgatgagtaccgtgtctaatcccgcatcattcctccg

SEQ ID NO: 145 - DNA, 45 bp, Synthetic construct
  source 1..45: mol_type = other DNA
acaggactcacgtgtccaaccatttgttctccctatgttcccacg

SEQ ID NO: 146 - DNA, 45 bp, Synthetic construct
  source 1..45: mol_type = other DNA
ccacacgcacacaaactcatgacgaattgcacttgtttttccggt

SEQ ID NO: 147 - DNA, 45 bp, Synthetic construct
  source 1..45: mol_type = other DNA
tcaacatcatgcactattgtccaaacgcgctacttgcttcccacc

SEQ ID NO: 148 - DNA, 45 bp, Synthetic construct
  source 1..45: mol_type = other DNA
ccacaaccccgacatttcactctattcatcgatcctgctgcgagg

SEQ ID NO: 149 - DNA, 45 bp, Synthetic construct
  source 1..45: mol_type = other DNA
acaacaattacccgtagtccagcatccgacgttttcctgccctcg

SEQ ID NO: 150 - DNA, 45 bp, Synthetic construct
  source 1..45: mol_type = other DNA
cgtgtccagaccgattttattccaaactgctgcccctactacgcg

SEQ ID NO: 151 - DNA, 45 bp, Synthetic construct
  source 1..45: mol_type = other DNA
caacacccacaaccttcttgtcaaccttttcatcgcgcgaatttg

SEQ ID NO: 152 - DNA, 113 bp, Synthetic construct
  source 1..113: mol_type = other DNA
agggcagcaggcagaagtatgcaaagcatgcatctcaattagtcagcaaccaatccactcaggattggttgctgactaattgagatgcatgctttgcatacttctgcctgctg

SEQ ID NO: 153 - DNA, 133 bp, Synthetic construct
  source 1..133: mol_type = other DNA
agggccaggctccccagcaggcagaagtatgcaaagcatgcatctcaattagtcagcaaccaatccactcaggattggttgctgactaattgagatgcatgctttgcatacttctgcctgctggggagcctgg

SEQ ID NO: 154 - DNA, 143 bp, Synthetic construct
  source 1..143: mol_type = other DNA
agggccaggctccccagcaggcagaagtatgcaaagcatgcatctcaattagtcagcaaccacatccattaactcataatggatgtggttgctgactaattgagatgcatgctttgcatacttctgcctgctggggagcctgg

SEQ ID NO: 155 - DNA, 109 bp, Synthetic construct
  source 1..109: mol_type = other DNA
agggctggggactttccagcctggggactttccagctgggactttccaggatccactcaggatcctggaaagtcccagctggaaagtccccaggctggaaagtccccag

SEQ ID NO: 156 - DNA, 111 bp, Synthetic construct
  source 1..111: mol_type = other DNA
agggctggggactttccagctggggactttccagctgggactttccaggagatccactcaggatctcctggaaagtcccagctggaaagtccccagctggaaagtccccag

SEQ ID NO: 157 - DNA, 18 bp, Synthetic construct
  source 1..18: mol_type = other DNA
atccagagtgacgcagca

SEQ ID NO: 158 - DNA, 18 bp, Synthetic construct
  source 1..18: mol_type = other DNA
tggacacggtggcttagt

SEQ ID NO: 159 - DNA, 105 bp, Synthetic construct
  source 1..105: mol_type = other DNA
agggagagagaaaatccagagtgacgcagcaccgcctgtgtcttacctaatgttgcgtcatctctgtgcgtcacgatggacacggtggcttagtaaaatctctct

SEQ ID NO: 160 - DNA, 105 bp, Synthetic construct
  source 1..105: mol_type = other DNA
agggagagagaaaatccagagtgacgcagcagcacaccacatcatactgtgtccaaccgttttgcgagtcctcccgtggacacggtggcttagtaaaatctctct

SEQ ID NO: 161 - DNA, 105 bp, Synthetic construct
  source 1..105: mol_type = other DNA
agggagagagaaaatccagagtgacgcagcatggtgtgtgtgcttatccctttctttggtcggttgctgcgttttgtggacacggtggcttagtaaaatctctct

SEQ ID NO: 162 - DNA, 105 bp, Synthetic construct
  source 1..105: mol_type = other DNA
agggagagagaaaatccagagtgacgcagcacaaaccacgacataccttttccgttccaggcaggtctttattccgtggacacggtggcttagtaaaatctctct

SEQ ID NO: 163 - DNA, 105 bp, Synthetic construct
  source 1..105: mol_type = other DNA
agggagagagaaaatccagagtgacgcagcaccccaccgctcaccatagtcactctcattgtccaacctctcactctggacacggtggcttagtaaaatctctct

SEQ ID NO: 164 - DNA, 105 bp, Synthetic construct
  source 1..105: mol_type = other DNA
agggagagagaaaatccagagtgacgcagcaccacacatccaaccgtaaatgctccttgtccagcaacccttaccgtggacacggtggcttagtaaaatctctct

SEQ ID NO: 165 - DNA, 105 bp, Synthetic construct
  source 1..105: mol_type = other DNA
agggagagagaaaatccagagtgacgcagcacaacacacatttcctcccccggcactgctggtcgattcgcgcggttggacacggtggcttagtaaaatctctct

SEQ ID NO: 166 - DNA, 105 bp, Synthetic construct
  source 1..105: mol_type = other DNA
agggagagagaaaatccagagtgacgcagcaggttatgtgggtggtgctgctgtgatggtgatgcgtccgatggggtggacacggtggcttagtaaaatctctct

SEQ ID NO: 167 - DNA, 105 bp, Synthetic construct
  source 1..105: mol_type = other DNA
agggagagagaaaatccagagtgacgcagcacacaactgaacacattgctgcacgtcttgatccctagctggttgctggacacggtggcttagtaaaatctctct

SEQ ID NO: 168 - DNA, 105 bp, Synthetic construct
  source 1..105: mol_type = other DNA
agggagagagaaaatccagagtgacgcagcaacaacgcctctcttcttcttgccctgagaacacacacactacccgtggacacggtggcttagtaaaatctctct

SEQ ID NO: 169 - DNA, 105 bp, Synthetic construct
  source 1..105: mol_type = other DNA
agggagagagaaaatccagagtgacgcagcaacacacaccatgcttctttgccctttctctcttttgcttcccctgtggacacggtggcttagtaaaatctctct

SEQ ID NO: 170 - DNA, 105 bp, Synthetic construct
  source 1..105: mol_type = other DNA
agggagagagaaaatccagagtgacgcagcaacaacaattacccgtagtccagcatccgacgttctcctgccctcgtggacacggtggcttagtaaaatctctct

SEQ ID NO: 171 - DNA, 16 bp, Synthetic construct
  source 1..16: mol_type = other DNA
tactggttgcaggatt

SEQ ID NO: 172 - DNA, 16 bp, Synthetic construct
  source 1..16: mol_type = other DNA
taagcactttggaaag

SEQ ID NO: 173 - DNA, 1801 bp, Synthetic construct
  source 1..1801: mol_type = other DNA
ggtctcgccctgatttaaatcgtcgaccgttacataacttacggtaaatggcccgcctggctgaccgcccaacgacccccgcccattgacgtcaataatgacgtatgttcccatagtaacgccaatagggactttccattgacgtcaatgggtggagtatttacggtaaactgcccacttggcagtacatcaagtgtatcatatgccaagtacgccccctattgacgtcaatgacggtaaatggcccgcctggcattatgcccagtacatgaccttatgggactttcctacttggcagtacatctacgtattagtcatcgctattaccatggtgatgcggttttggcagtacatcaatgggcgtggatagcggtttgactcacggggatttccaagtctccaccccattgacgtcaatgggagtttgttttggcaccaaaatcaacgggactttccaaaatgtcgtaacaactccgccccattgacgcaaatgggcggtaggcgtgtacggtgggaggtctatataagcagagctcgtttagtgaaccgtcagatcgcctggagacgccatccacgctgttttgacctccatagaagacaccgggaccgatccagcctccggactctagaggatccggtactcgaggaactgaaaaaccagaaagttaactggtaagtttagtctttttgtcttttatttcaggtcccggatccggtggtggtgcaaatcaaagaactgctcctcagtggatgttgcctttacttctaggcctgtacggaagtgttacttctgctctaaaagctgcggaattgtacccgcggcccgggatccaccggtcgccaccatggtgagcaagggcgaggagctgttcaccggggtggtgcccatcctggtcgagctggacggcgacgtaaacggccacaagttcagcgtgtccggcgagggcgagggcgatgccacctacggcaagctgaccctgaagttcatctgcaccaccggcaagctgcccgtgccctggcccaccctcgtgaccaccctgacctacggcgtgcagtgcttcagccgctaccccgaccacatgaagcagcacgacttcttcaagtccgccatgcccgaaggctacgtccaggagcgcaccatcttcttcaaggacgacggcaactacaagacccgcgccgaggtgaagttcgagggcgacaccctggtgaaccgcatcgagctgaagggcatcgacttcaaggaggacggcaacatcctggggcacaagctggagtacaactacaacagccacaacgtctatatcatggccgacaagcagaagaacggcatcaaggtgaacttcaagatccgccacaacatcgaggacggcagcgtgcagctcgccgaccactaccagcagaacacccccatcggcgacggccccgtgctgctgcccgacaaccactacctgagcacccagtccgccctgagcaaagaccccaacgagaagcgcgatcacatggtcctgctggagttcgtgaccgccgccgggatcactctcggcatggacgagctgtacaagtaaagcggccgcggggatccagacatgataagatacattgatgagtttggacaaaccacaactagaatgcagtgaaaaaaatgctttatttgtgaaatttgtgatgctattgctttatttgtaaccattataagctgcaataaacaagttaacaacaacaattgcattcattttatgtttcaggttcagggggaggtgtgggaggttttttagtcgaccatttaaatcggtctcgaggg

SEQ ID NO: 174 - DNA, 1857 bp, Synthetic construct
  source 1..1857: mol_type = other DNA
gcgtataatggactattgtgtgctgataggtctcgccctgatttaaatcgtcgaccgttacataacttacggtaaatggcccgcctggctgaccgcccaacgacccccgcccattgacgtcaataatgacgtatgttcccatagtaacgccaatagggactttccattgacgtcaatgggtggagtatttacggtaaactgcccacttggcagtacatcaagtgtatcatatgccaagtacgccccctattgacgtcaatgacggtaaatggcccgcctggcattatgcccagtacatgaccttatgggactttcctacttggcagtacatctacgtattagtcatcgctattaccatggtgatgcggttttggcagtacatcaatgggcgtggatagcggtttgactcacggggatttccaagtctccaccccattgacgtcaatgggagtttgttttggcaccaaaatcaacgggactttccaaaatgtcgtaacaactccgccccattgacgcaaatgggcggtaggcgtgtacggtgggaggtctatataagcagagctcgtttagtgaaccgtcagatcgcctggagacgccatccacgctgttttgacctccatagaagacaccgggaccgatccagcctccggactctagaggatccggtactcgaggaactgaaaaaccagaaagttaactggtaagtttagtctttttgtcttttatttcaggtcccggatccggtggtggtgcaaatcaaagaactgctcctcagtggatgttgcctttacttctaggcctgtacggaagtgttacttctgctctaaaagctgcggaattgtacccgcggcccgggatccaccggtcgccaccatggtgagcaagggcgaggagctgttcaccggggtggtgcccatcctggtcgagctggacggcgacgtaaacggccacaagttcagcgtgtccggcgagggcgagggcgatgccacctacggcaagctgaccctgaagttcatctgcaccaccggcaagctgcccgtgccctggcccaccctcgtgaccaccctgacctacggcgtgcagtgcttcagccgctaccccgaccacatgaagcagcacgacttcttcaagtccgccatgcccgaaggctacgtccaggagcgcaccatcttcttcaaggacgacggcaactacaagacccgcgccgaggtgaagttcgagggcgacaccctggtgaaccgcatcgagctgaagggcatcgacttcaaggaggacggcaacatcctggggcacaagctggagtacaactacaacagccacaacgtctatatcatggccgacaagcagaagaacggcatcaaggtgaacttcaagatccgccacaacatcgaggacggcagcgtgcagctcgccgaccactaccagcagaacacccccatcggcgacggccccgtgctgctgcccgacaaccactacctgagcacccagtccgccctgagcaaagaccccaacgagaagcgcgatcacatggtcctgctggagttcgtgaccgccgccgggatcactctcggcatggacgagctgtacaagtaaagcggccgcggggatccagacatgataagatacattgatgagtttggacaaaccacaactagaatgcagtgaaaaaaatgctttatttgtgaaatttgtgatgctattgctttatttgtaaccattataagctgcaataaacaagttaacaacaacaattgcattcattttatgtttcaggttcagggggaggtgtgggaggttttttagtcgaccatttaaatcggtctcgagggtatcagcacacaattgcccattatacgc

SEQ ID NO: 175 - DNA, 18 bp, Synthetic construct
  source 1..18: mol_type = other DNA
atccagagtgacgcagca

SEQ ID NO: 176 - DNA, 18 bp, Synthetic construct
  source 1..18: mol_type = other DNA
actaagccaccgtgtcca